European Patent Specification EP 3 508 589 B1, published March 1, 2023. Title: Diagnostic method. Applicant: CLINICAL GENOMICS PTY. LTD. COMMONWEALTH SCIENTIFIC AND INDUSTRIAL RESEARCH ORGANISATION ROSS, Jason DREW, Horace BUCKLEY, Michael MOLLOY, Peter MITCHELL, Susan DUESING, Konsta BROWN, Glenn. The sequence listing filed with the application follows.

SEQUENCE LISTING (82 sequences)

SEQ ID NO: 1 - DNA, 21 bp, Artificial
  CG linker-upper
cgcgtatcaccgactgccctt

SEQ ID NO: 2 - DNA, 17 bp, Artificial
  CG linker-lower
gggcagtcggtgatacg

SEQ ID NO: 3 - DNA, 21 bp, Artificial
  CA linker
cagcaatcaccgactgccctt

SEQ ID NO: 4 - DNA, 17 bp, Artificial
  CA linker
gggcagtcggtgattgc

SEQ ID NO: 5 - DNA, 11 bp, Artificial
  CG competitor
acagagtcgta

SEQ ID NO: 6 - DNA, 12 bp, Artificial
  CG competitor
cgtacgactctg

SEQ ID NO: 7 - DNA, 11 bp, Artificial
  CA competitor
agtgatcagca

SEQ ID NO: 8 - DNA, 12 bp, Artificial
  CA competitor
catgctgatcac

SEQ ID NO: 9 - DNA, 29 bp, Artificial
  P2-N6 primer
  misc_feature (24)..(29): n is a, c, g, or t
ctgccccgggttcctcattctctnnnnnn

SEQ ID NO: 10 - DNA, 21 bp, Artificial
  P2-long primer
ctgccccgggttcctcattct

SEQ ID NO: 11 - DNA, 24 bp, Artificial
  SolP2-AB linker
cctaccccacattcctcattctct

SEQ ID NO: 12 - DNA, 25 bp, Artificial
  SolP2-BP linker
ttggatggggtgtaaggagtaagag

SEQ ID NO: 13 - DNA, 41 bp, Artificial
  SolP1 AM linker
mmamtamgmmtmmgmtttmmtmtmtatgggmagtmggtgat

SEQ ID NO: 14 - DNA, 44 bp, Artificial
  SolP1 BC linker
cggtgatgcggaggcgaaaggagagatacccgtcagccactaat

SEQ ID NO: 15 - DNA, 251 bp, human
gatgggtgttgggacatggagtccccagcctgtgctgctgacgccctgtggtggctagccgctctttagacaccagacgctgccttccacttcctcctctcacttcttattcgggcaccactgacgacagagacttcggctgggccattcccgcctctcctaccgcctggcagccatggtaacagcctgggggatggtccctaagatggggtcagagaacggctgagcatggccatccccccagccctgaa

SEQ ID NO: 16 - DNA, 299 bp, human
caggaagctgcagcagaaggaggaggcggcggccaccccggaccccgccgcccggactcccgactcggaagtcgcgcccgccgctccggtcccgaccccgggaccccctgccgcagccgccacccctgggcccccagcggacgagctgtacgcggcgctggaggactatcaccctgccgagctgtaccgcgcgctcgccgtgtccgggggcaccctgccccgccgaaaggtgcgtcccccgcccgccttcaggatctgctcagcccctctccgactccctacagggcctgctgactccg

SEQ ID NO: 17 - DNA, 258 bp, human
gacagagacagccccaggcaagttgaaggtccgagagcccccggtgggagaagcgggccggtggctgcgccgcgtgcgttctcactctgaggaagtgcgtggggagccgctgactccggatagcacacccttccgaggggactccccgattcctgggctgggggcctgccgcctggccccacgtctgacgtacggggcgcgagggccactgctccctggacttctgtcggaaccggacgcagtgggaggggtcgcagg

SEQ ID NO: 18 - DNA, 233 bp, human
aacttgcatgcagtcaaacaggaaagctggcgcgggggggatggtgtgcggaggaagggaccccgaagtttccaggtcatccctggtctcgaggagcgcgcggagtggagccgttccctcgcgggcccgacccaggctcccccctcctgccaccctttcccctccgtccttcccagaccacgcagcaagacccgccgagggcgaagaagttgggagtgacttcaggggcctct

SEQ ID NO: 19 - DNA, 221 bp, human
ccgcaggactgggaatccagtggccggcgtcccagcattttcggacgcgttccgtgcctcccccagtatccccttgagggatcgcctactgcgattccacgtagtgtcggttacctcgccctagccgcagggagcatcaaacaaaagaacttttgcaaacttttctctctggacactcgcgggtctcttaaatctggcccccatctccccagaacttgcat

SEQ ID NO: 20 - DNA, 237 bp, human
aaaggaggctcggtccaccaatgcgcgatcgtagcctacagggacccccaacgaaccccggcccagagaatgcacctggccgtgccacgcgcgacccccgaggggcaggcggacgggtccaggcgcggacaaaggggcctctcggggcgcccaagctcggggcgggacgccgggagcggagctggccgggaactcaccttcgcagcggcccggctgtgctcctcgtggagcagaagg

SEQ ID NO: 21 - DNA, 254 bp, human
tgcgttacataatggaggattaaagaaaacagtgtcccttggcttaaaacaaatggtgtcctcttagtctcccgtcccagtgggcgttagatgtcggggcaggcggctgcacacttaattctccgcgggggcattggcctgtctgccggtccaaatcatccattttccttggtctgactgcaaggtcggtgcttaaacttcggacggctggtgaattgtgcggcgggcgcggggccctgggaggcagccccctc

SEQ ID NO: 22 - DNA, 186 bp, human
gaacttgccgatgtggcaggtgtacagtccgtggctaggcaggaaggcggggtgttgcagcggcgccccggcggagggcccgtgcgcgccggggtggcccgcgggtggtggtggcgaagccttgggcgcaccgtcggggctcgtggctgtctccgccagcgaccagatcttgggcttgccgtgcgg

SEQ ID NO: 23 - DNA, 193 bp, human
gaccgaggccttgtctccattgagtgcccccggggcaatagcgaccggcggctgcggtggtggaggtgcaggaaggtgagggccatggggcgcggcgtggggagcgccaacgcccaggaaggagcgcatgttgagcagggagccctgtgcgaggaatgcgctgttggtccagttggagaacttgccgatgtgg

SEQ ID NO: 24 - DNA, 191 bp, human
ggagtccggtgtgctggagagccgcagcggggtgaactcccggccccgtctctgcgtaggaggtggttcgcaaagtggccccgggagccgggactggtacccggttccccacggcaccgtccggagctctccagccacgaggcgcagaagtggcctgccagcgccttcccaggctcagggaggcgaggagg

SEQ ID NO: 25 - DNA, 166 bp, human
gggcgccgagtggaaactgctcacagagtcggagaagcggccgttcatcgacgaggccaagcgtctacgcgccatgcacatgaaggagcaccccgactacaagtaccggccgcggcgcaagcccaagacgctgctcaagaaggacaagttcgccttcccggtgccc

SEQ ID NO: 26 - DNA, 270 bp, human
tgagagccccctttggcacttggcagcacgcggcggcgggctcctcggctcaacttcgaggagtctccgcgacgcaacttttggggacgctttgcatttaagagagaacgaccgaggaggaggagcgctctgcccggccgccgctacctgcggggagctcaccagcaaacgccactgcagacgaaggacccaaagaacgtaaagggcaaactgccgccgcggggagggggcaccgccgagaagttagagtgtcccagagacaacctgctc

SEQ ID NO: 27 - DNA, 311 bp, human
gcggtcagttacatgtgctggtgtccagccgctgcctctctttccccggtcggagcgcgggggtgcgtgtgccctcactctcacgaatacagacggagagcttcccagaaggaaaaacaaattcgtcataatgttcagcgcagccgagagtttccaacaagaaagcagctccagtcgtggcatgatgactcagggtggcgttttaaacgctgaataaacccattccttagctctttaataaatcgctaataacagcaaaaacagccttctccccgaaccgcgccacaccaaaggcttcccaagttgggctg

SEQ ID NO: 28 - DNA, 253 bp, human
atagcagggtttacagggcaaagagaggagaacctggaaatcgtgtcctggggggcaagagtgcgttgcccagtcacaagtgtgctgtagaggtgggagaggacaaggacccatttccacatttcaaccctccgtttctatcgctgcccctggaggactcagctgctaacgccgagctcgtttccacgcggctctggtcctagtcggggaatccgggtggccgcgcgacgcgagagaactgctgggatgcgtg

SEQ ID NO: 29 - DNA, 222 bp, human
gatgcgtggccctggtatgggcgcacccagcgtccggggcgcaggttctctcagcccagcttctcctcccactcactcgctcggatctcctccctccttcacatcccccgcccccgggaccgcgaggctccctccccgcaccggccagtgagtacacaaagccgcgggtgaggggaagcttcgcaggcgtgcacggagcagtgagatcactggcgttataaa

SEQ ID NO: 30 - DNA, 181 bp, human
gctgctgaaggagtgagagggaccttagagcagagcgggcggtgcctgcgcagtgcgtgattacgcgagccgggcgtggcccagggttccggcgggtaagagcaggagtgtgcgcaggcgcaaagattgcgctctccccctctcctcgcctagagaccagaagcgtccctagttactagtt

SEQ ID NO: 31 - DNA, 280 bp, human
gttttgggtggtttgggagtccgagctcgagggctgggccaggaagggcaggcgaggcgggcggctccgacgcgggtcgcgaaggcccagccgcgtcctctgtccccaggacgactacatttcccagaggccagcggggcgcgcgtactcgagtctgcggggcggaggccgcggctcggggctgctgggcgttcggggcggcttggggcggcgggaccactggagtgagctgtgggagagatgggggtgtgcctgtgtgtaaaagatctgtcagagtgtg

SEQ ID NO: 32 - DNA, 253 bp, human
ggggagggggaggaggccagttgaaaagtagaggccgaggacagagttagacactcgttgtctaacggccctgccggaggggctccgcctgtcagactgcgtcaccctctcgccaagggtcccccagacgggcgggggctccttgcggccggctagctactctccccgcctccctgcgccctcgccctccgccccgctgtacccgcagagcgcgcggcccagcgcagccccttttggcaccgaggtttccagg

SEQ ID NO: 33 - DNA, 251 bp, human
ggtttcaggctgcctaggaccggaaccagggatcgcaccgcagcccaaggtaccagtttcgggcgggcggcctggcccggcagggagatgaggtcccctttcttaacagcaagctaacgcggcggtcccctggagctgctcagcgtcccagcttctaaccagctcctatggaatccaggtgcggcttaaatctcgcacactggtcccctaaactttcaaaaccacgtttatgggcaaagccctgccggctg

SEQ ID NO: 34 - DNA, 205 bp, human
ggctccctcagcgatgtggaggaccttcaagaggtggagatgttggaatgtgacgggttgaaaatggattcgaacaaggaatttgtgacttccaacgagagcaccgaggagagctccaactgcgagaatgggtctccccagaagggccgcggcggcctgggcaagaggaggaaggcgcccaccaagaagagccccctgagcgggg

SEQ ID NO: 35 - DNA, 240 bp, human
gaggaaggcgcccaccaagaagagccccctgagcggggtcagccaggaggggaagcaggtccagcgcaacgccgccaacgcgcgagagcgggcccgcatgcgagtgctgagcaaggccttctccagactcaagaccaccctgccctgggtgccccccgacaccaagctctccaagctggacacgctcaggctggcgtccagctacatcgcccacttgaggcagatcctggctaacgacaa

SEQ ID NO: 36 - DNA, 281 bp, human
gggatccctcctctgtgccagctcaacacacttgcaaacttttaattgggctgccacgtcaaaccctcgcataaatcactcccgctccgggggctggtagggcagagagcgagggccgtgtctagaccgcccgcctccggtccctggaggctctaggcccgcggtggtcgagatgtgtaagtcaccgccgcgcccacacccccactcccagccccgcgcgcactcgcgcccaccgcaggcgggagtgcgggcgcgcctggactgcagctgcagccccggga

SEQ ID NO: 37 - DNA, 225 bp, human
aggctttcaaggggaaactctgactcgttgtctgcatacctccgccctccgcatcctcccgccctcccccgccctttccaagtttggaaacactatgggacacgtcggagtgctctgcagccccgacatgggcagaatttgcagatctccggcgatcaaagcaggagctgtccagtcccgcctcacctgtgccctgtaggccacttgtagggtggagggctccag

SEQ ID NO: 38 - DNA, 205 bp, human
ggaggcaccctagggccagggaaacttttgccgtataaatagggcagatccgggctttattattttagcaccacggcagcaggaggtttcggctaagttggaggtactggccacgactgcatgcccgcgcccgccaggtgatacctccgccggtgacccaggggctctgcgacacaaggagtctgcatgtctaagtgctagacat

SEQ ID NO: 39 - DNA, 198 bp, human
gagggaggacatggaggcagccacctagctcagcggagacgcggagcccacagcagcgccctccggagccctaacacgtcgctgccaccatccgcgccgggactccgcagccgagctcggccgcccgcaggacgctccaggagcgtcgcggaccgggcggcacgggacgctgcggggctgagctcaagagcccaggtt

SEQ ID NO: 40 - DNA, 282 bp, human
agtctgttactcggtctggctgaccccgccggtgtctctgtgcatccatgctacctttccctattacccacccccttcccagatccgagcagtccgccggcccgcgcggacccagagcaagaagagggcgaggaagaagatgcctcggcccggccgcaacacgtacagcgaccagaagccgccctactcgtacatctcgctgaccgctatggccatccagagctctcccgagaagatgctgccgctgagcgagatctacaagttcatcatggaccgcttccc

SEQ ID NO: 41 - DNA, 211 bp, human
gagttcatgttcgaggagggctcctttcggcggcggccgcgcggcttccgaaggaaatgccaggcgctcaagcccatgtacagcatgatgaacgggctcggcttcaaccacctcccggacacctacggcttccagggctcggccggcggcctctcgtgcccgcccaacagcctggcgctggagggcggcctgggcatgatgaacggccact

SEQ ID NO: 42 - DNA, 320 bp, human
gtccggcccgtccaaggccaagaagaccaacgccggcatccggcgcccggagaagccgccctattcctacatcgcgctcatcgtcatggccatccagagttcacccaccaagcgcctgacgctgagcgagatctaccagttcctgcagagccgcttccccttcttccggggctcctaccagggctggaagaactccgtgcgccacaacctctcgctcaacgagtgcttcatcaagctacccaagggccttgggcggcccggcaagggccactactggaccatcgacccggccagcgagttcatgttcgaggagggctcct

SEQ ID NO: 43 - DNA, 316 bp, human
ccctgcccagccactcggtgccccacctgccttccaacggcggccactcgtacatgggcggctgcggcggcgcggcggccggcgagtacccgcaccacgacagctcggtgcccgcctccccgctgctgcccaccggcgccggtggggtcatggagccgcacgccgtctactcgggctcggcggcggcctggccgccctcggcgtccgcggcgctcaacagcggcgcctcttatatcaagcagcagcccctgtccccctgtaaccccgcggccaaccccctgtccggcagcctctccacgcactccctggagcagcc

SEQ ID NO: 44 - DNA, 212 bp, human
ggttgggcccgggatcagagctttgcttggaagttctctgggtggcagagactcgggcaaccggagcctgagcctcccgcggggaagagctcggactccggaggtcgcgccgccttgggcttgaattcagtccttccttactactcgtggctttgcttacatcatttaactctccatttccttgtctatacagtgggctcataaggaggcgg

SEQ ID NO: 45 - DNA, 187 bp, human
cttccagggaggcccagggaggcagcggagagcgaagtcctgctcggcggagagacctcgaggagagtatggggaaaggaatgaatgctgcggagcgcccctctgggctccacccaagcctcggaggcgggacggtgggctccgtcccgaccccttaggcagctggaccgatacctcctggatcaga

SEQ ID NO: 46 - DNA, 205 bp, human
gaagattccaagaggaatggagggcttgtggctccagctcggacggtctctggggcaaggaggtgcaggaggctgcgctgttggatttctcctcggggtgagcagggccgggctgtcctgccggctctggagcgcatatgccgagccagcgcgcacttgggtagggctaactgcgttcagctttggcaggagctctgctcttcct

SEQ ID NO: 47 - DNA, 102 bp, human
agagtaagagagagcagcccatctaatagagtgtcccggaggccagcgccagcgggtgctgtaaggagcccggcggcggcaggtgggaattgattgagctgg

SEQ ID NO: 48 - DNA, 165 bp, human
gtgcagctcaggcaggtctagtgcatggcagcgccgtatttacctgtgtttgtgtcaatcccagcgaggcggccagctcggcgcgttccggcaaggcgaggtactgagtcttctgaaaccttctctgtaatgcggccagctgaaagctggaataaatagtcctgg

SEQ ID NO: 49 - DNA, 180 bp, human
ctgcccagccttccccctgtccatgtacctggctggttggtggcgcttgggacgcggttgtaggcgccgccgtactggtggtaggagctagcgtagctatagtcggcataagctttggctgggtagctcccggcggagccgttcacgccgtgatactgatactggtaggggttgagagct

SEQ ID NO: 50 - DNA, 164 bp, human
gtgaccagcactttgtactgctggggccgctccagggagaagactctcccttccaccgcttttctccctcgccggtttcctggaccacccttcctccccaccgcccggttgcggtaactcagttaccgcgctgggctgcggttcccaggagggagggttcggtt

SEQ ID NO: 51 - DNA, 284 bp, human
ctggaatgggtgatctgggacgcggctcaattccctagagcataaggagggaattgcgctttttcttcttcattcgagaaatgatcggctcccgccagtctgcgtgctttcactcaacagcagctgcaagccctaggccagcgtcgcagaaacggccaggaaccccactttcctacccgggggccagcagcgatcgctggggctagcaagcgtgcagagggggaaagaaggaaatcggcttccttcccggacccctccttcctcttcctaccaggaagggaaaa

SEQ ID NO: 52 - DNA, 159 bp, human
aaagtgggaggggctcaaggacccagaggaaggacgtgtttcacaggcggaaagccgcggggacaatggcgagagcgaccgccctagccccgggcggacccgcaaccctcacactcgcgcgcccccgcgttagtgctcgaactggtctccgcctttccg

SEQ ID NO: 53 - DNA, 355 bp, human
agtgtgtcagtcactaggcagtgagacgccaggcttagggcgaaaaaagttttcctggaactcgggagctggtggggagtctctgtcacggactgagggttttttgtgtttttaaatgggagtctctgggtaaaggggcggggcgaggaggcgaacgagacaaccttagtattgtttgaattgaagcattgcgagggaacaatggcagaaaaaccgcgttttctcccaagtcctgttccggccctggaagagctgctccgggcgccacactgggatcctgttcgccgagcctgcccctccacgccggccgtgcacagccctgccgataccgtgggtgcagctggcgactgcactg

SEQ ID NO: 54 - DNA, 329 bp, human
gatggagtagccctgccctgtggcagccggggcccaggtggattcctcctgggaacgacccctccctcctcagcgcgcactgtgccagagcagtacacaggtacaaagggcaaacgtgttcatgatttcatttgaattctgttgtttttacatcgttctgccctgatgtaaaacaaaccaggattttaaaggcagtgagtgatgaggagctactcccacttggggaagagctgctaactttacttttccgctgctgttggttccggttcaaagctcggtttgggaagtaagaggaggactcggagactttgaccagagcactccaggcc

SEQ ID NO: 55 - DNA, 364 bp, human
agaaagctgaagtgacctgtgagactcctctccacctcacccgcggccaaaacgcccagcgccgggtctgggtttgcgaacggctcagcccaggccctgcgccagagcaccgcacccgggggcggacggccctgcagctccccagcctcttcccgcatcaactagctgacgcccgggcgcactggcttcccccgctcccgtttcgtattaattagttgacgttcgggcgtattggtttttttcgttttcgttttgtattaattagttgatgtttgggtgtattggttttttttgtttttgcccgcacgaaagccctgcccgacgtctgcagtcagcatcgcccgcactgcctagggagggtttg

SEQ ID NO: 56 - DNA, 205 bp, human
cccgcactgcctagggagggtttgcgccgagacccagtggccgagtgagccacagagtcgctggtcctggggacgctgtcttctaccgctccccaccgtcctcctctttcctgtatctcaccccggtaccccgcacccttctccccgctcggccccgcgcactctgctcagactttacaagcactttctcggggcacccaggact

SEQ ID NO: 57 - DNA, 304 bp, human
acaagcactttctcggggcacccaggactcgacgcctcctccgcgccgccagcggcgctcgccacccttggcacgccggagggaccgcctccggccccctgcgcggcgtttctcaggggactcccagcccatccctcacccagctgtccgggtcccgacgccttacctttgccgaactgggggacaccgaggctgagcccgaccaagagccagacggctaccgagcgcttcatgatcccgtctcccggacgtgaccccggctggtcaggggtcgtcgcggagggcagtgtagccgaggtggcag

SEQ ID NO: 58 - DNA, 309 bp, human
ggggactcccagcccatccctcacccagctgtccgggtcccgacgccttacctttgccgaactgggggacaccgaggctgagcccgaccaagagccagacggctaccgagcgcttcatgatcccgtctcccggacgtgaccccggctggtcaggggtcgtcgcggagggcagtgtagccgaggtggcagcgcagggcagcagcagactccgcccctactaaagaattcaagaagacgttctctttcctcagcgctttgttaaacaaattcttggagagggcgagagtggtgactaaagagaggagcctt

SEQ ID NO: 59 - DNA, 275 bp, human
gagagtggtgactaaagagaggagcctttcctccccttttgcctgcgctccggcgcgcggaggtgggtgagctccggggagccgccggcgggctcagccctccgctgcgggtgggtcccggcagaggcgcggcgggcggggcgcgggctcccgcggccgccccgggtctgctgcgcgggcaggcagacccaccggcagacaggcggaccgggcgctcggctgtcgctgttctccgcgcggcggctgcggggcttctgacttggagaacaatgaag

SEQ ID NO: 60 - DNA, 249 bp, human
actggttttctctcgggccagggcctccggggcaaccgtctccagcgcgcattcttggtgcaggtggaacagctttctgctccggtagggcttcacctatcgcgggagaggttaatctcggatctaaacctcgcagccgcagagcgggctaaaaccgctactccacctcttcccatttctcccctccccacctcaagacaaaaagtcccaggccgggcaggacctgatcacctctgcctcctcccactg

SEQ ID NO: 61 - DNA, 247 bp, human
ccctaccactccgggaactctgtgatcttcaggaccggcgggtttcaagtggcgctgttttcggtctctcctgaggtcgcaaccctcttcccacgaacaacagcccacaggctccgcagctcgccttggtctcaacaaccgcgcagtacttgggtgcttaagcgagtcccctaccacatagtccagggttgggggcgggggagatggggctgggaggggacagtggccaggagtagcggaaagagaa

SEQ ID NO: 62 - DNA, 229 bp, human
aaggaccttgtaagagaaagggagaaaagattttgtgtgtggagcgtgcctcgtaaggtttcgtgcttaggagaagttgggaggaggcagctcgcctagagtctttacggaccgaattcggagtttatttcgaacactatgcatcaagccaaagaaaagcggggccagtttgggtttgcgcctaacttaattccgatacgcgcgtcaaaatgttgtgtaggctggggcc

SEQ ID NO: 63 - DNA, 211 bp, human
gagggagagaaaagaatactgaaaataaagctggcggccgcgggctactgcctgcgtttgtgtgcgtgtgccctgggtgtgtggtgtttgtgcctgggcgtgcgatttaatggagcgcctctctgcctctccagtgcggccagagctcgcttcgcgcacccacccctgccgaggagcctacttgctgcagcccaatgcattgtgtaagacg

SEQ ID NO: 64 - DNA, 254 bp, human
ccgaggagcctacttgctgcagcccaatgcattgtgtaagacgcgacctgttatggccaccactacttccgggttctagcattctggtcggaatccacctctccgcctgtgcaacacacactttacacacgcacggggactgcaagcgggcagcatcgatcgtggctcctttaagacaaactcagacagacattttttttaaccctccttctctaatctccttccagtgcagcacttgcaaagagggagagaga

SEQ ID NO: 65 - DNA, 195 bp, human
cagcctcagaaccccctgctgggaaacatctgtcgctctaggcccttgacgtcctgaggttagagagcagcggtactactaggagggacgccggcttggctaggacaccctgcactccctggggtcaggaacgggaaggaatggtcagaaacagatgatcagccacaatgatagatggtcagagacagaaatttt

SEQ ID NO: 66 - DNA, 300 bp, human
caacttttggacacatctgggcagttgctaagggctcttgccaagcgtctaggtaagcctttggcaaacagctacaggggtcgtttttgctaatgtaggactttgggaacggtgctctggcacacaatttgggtaaacttatgcgcgcataaggatgggagggagcttggtcaaagcggggcttggcaaatttctaggaaccttcggcacagatccggagagggacctttaaacaaacagctcgagggggccatttgggaagtgattggggcaggagggaagcagagagcgcatcttttt

SEQ ID NO: 67 - DNA, 172 bp, human
ggcgaggaagctccataaaagccctgtcgcgacccgctctctgcaccccatccgctggctctcacccctcggagacgctcgcccgacagcatagtacttgccgcccagccacgcccgcgcgccagccaccgtgagtgctacgacccgtctgtctaggggtgggagcgaacgg

SEQ ID NO: 68 - DNA, 193 bp, human
ttaccttttagcagatatggagggagaacccgggaccgctatcccaaggcagctggcggtctccctgcgggtcgccgccttgaggcccaggaagcggtgcgcggtaggaaggtttccccggcagcgccatcgagtgaggaatccctggagctctagagccccgcgccctgccacctccctggattcttgggct

SEQ ID NO: 69 - DNA, 205 bp, human
gggagaaaagtgacccagcaggaagaacttccaattcggttttgaatgctaaactggcggggcccccaccttgcactctcgccgcgcgcttcttggtccctgagacttcgaacgaagttgcgcgaagttttcaggtggagcagaggggcaggtcccgaccggacggcgcccggagcccgcaaggtggtgctagccactcctgggt

SEQ ID NO: 70 - DNA, 174 bp, human
acaaatggatggatgagtgaatgaatgaacgaaggaacaagtgaccgctcgaccttctacagcgacagcggcgcaggcgctcccgcaccaacagccccccaccccgccaccgccagagggcgcagacaggccgggtcccgagtgtctgtcccaggcccccgccccacaggatcc

SEQ ID NO: 71 - DNA, 260 bp, human
tcgtcctcttgtgcagaccaggctggccgtgcaccagcgagtgtgcaccgagaccccaagggcgtggggtctccgcgcccgggctctatctgtccccgaccacccccgagccctccccgggctcaccatgccgcggtacagctcctccaggcgcccgtcgatccacttctccacgtccagccgccgctgcagctcccgccggtcatacttgacggtgacgcgcgcgtgccgcttctgcagccccccgggactgccccctg

SEQ ID NO: 72 - DNA, 17 bp, human
cggaagtcgcgttcgtc

SEQ ID NO: 73 - DNA, 20 bp, human
gcgtacaactcgtccgctaa

SEQ ID NO: 74 - DNA, 23 bp, human
gaatgtatttggtcgtgttacgc

SEQ ID NO: 75 - DNA, 14 bp, human
cccgacgtcccgcc

SEQ ID NO: 76 - DNA, 23 bp, human
tttagtattttcggacgcgtttc

SEQ ID NO: 77 - DNA, 26 bp, human
gaaataaccgacactacgtaaaatcg

SEQ ID NO: 78 - DNA, 21 bp, human
cggagacgttcgttcgatagt

SEQ ID NO: 79 - DNA, 22 bp, human
caaacgaatcgtaacactcacg

SEQ ID NO: 80 - DNA, 23 bp, human
ctaaacccgtccgcctacccctc

SEQ ID NO: 81 - DNA, 20 bp, human
cggattttcgattcggaagt

SEQ ID NO: 82 - DNA, 250 bp, human
tagcgcaggatgagggaggcagcccatcctcaccgccggtctcggtccgcgagacgcggggacagcgcggtgcgcggcccgcatgcaggggtgaccggagggccgtcccccccacgacccggaaagaaggagagcctcccgttaggcccctgtgggtgctccttggccgaggagctcggtcttcgctctcccaccctccccctttctactcccaagcaggagagcgtgcagccctagcctgcacaaggcg